European Patent Application EP 4 286 499 A1, published December 6, 2023. Title: DISHWASHING DETERGENT COMPOSITION COMPRISING XYLANASE AND SULPHONATED CARBOXYLATE POLYMER. Applicant: THE PROCTER & GAMBLE COMPANY. The sequence listing filed with the application follows.

SEQUENCE LISTING (1 sequence)

SEQ ID NO: 1 - protein, 248 aa, Bacillus agaradhaerens
MRQKKLTFILAFLVCFALTLPAEIIQAQIVTDNSIGNHDGYDYEFWKDSGGSGTMILNHGGTFSAQWNNVNNILFRKGKKFNETQTHQQVGNMSINYGANFQPNGNAYLCVYGWTVDPLVEYYIVDSWGNWRPPGATPKGTITVDGGTYDIYETLRVNQPSIKGIATFKQYWSVRRSKRTSGTISVSNHFRAWENLGMNMGKMYEVALTVEGYQSSGSANVYSNTLRINGNPLSTISNDKSITLDKNN